European Patent Specification EP 4 139 299 B1, published December 17, 2025. Title: KRAS G12D Protein Inhibitors. Applicant: Taiho Pharmaceutical Co., Ltd. The sequence listing filed with the application follows.

SEQUENCE LISTING (4 sequences)

SEQ ID NO: 1 - protein, 188 aa, Artificial
  Synthetic protein
MASSHHHHHHSSENLYFQGMTEYKLVVVGADGVGKSALTIQLIQNHFVDEYDPTIEDSYRKQVVIDGETCLLDILDTAGQEEYSAMRDQYMRTGEGFLCVFAINNTKSFEDIHHYREQIKRVKDSEDVPMVLVGNKCDLPSRTVDTKQAQDLARSYGIPFIETSAKTRQGVDDAFYTLVREIRKHKEK

SEQ ID NO: 2 - protein, 487 aa, Artificial
  Synthetic protein
GEEQMRLPSADVYRFAEPDSEENIIFEENMQPKAGIPIIKAGTVIKLIERLTYHMYADPNFVRTFLTTYRSFCKPQELLSLIIERFEIPEPEPTEADRIAIENGDQPLSAELKRFRKEYIQPVQLRVLNVCRHWVEHHFYDFERDAYLLQRMEEFIGTVRGKAMKKWVESITKIIQRKKIARDNGPGHNITFQSSPPTVEWHISRPGHIETFDLLTLHPIEIARQLTLLESDLYRAVQPSELVGSVWTKEDKEINSPNLLKMIRHTTNLTLWFEKCIVETENLEERVAVVSRIIEILQVFQELNNFNGVLEVVSAMNSSPVYRLDHTFEQIPSRQKKILEEAHELSEDHYKKYLAKLRSINPPCVPFFGIYLTNILKTEEGNPEVLKRHGKELINFSKRRKVAEITGEIQQYQNQPYCLRVESDIKRFFENLNPMGNSMEKEFTDYLFNKSLEIEPRNPKPLPRFPKKYSYPLKSPGVRPSNPRPGT

SEQ ID NO: 3 - DNA, 567 bp, Artificial
  Synthetic DNA
atggcaagcagccatcatcatcatcatcatagcagcgaaaacctgtattttcagggcatgaccgaatataaactggttgttgttggtgcagatggtgttggtaaaagcgcactgaccattcagctgattcagaatcattttgtggatgagtatgatccgaccatcgaagatagctatcgtaaacaggttgtgattgatggtgaaacctgtctgctggatattctggataccgcaggtcaagaggaatatagcgcaatgcgtgatcagtatatgcgtaccggtgaaggttttctgtgtgtttttgcaatcaacaataccaaaagcttcgaggatatccatcattatcgcgagcagattaaacgtgtgaaagatagcgaagatgttccgatggttctggttggtaataaatgtgatctgccgagccgtaccgttgataccaaacaggcacaggatctggcacgtagctatggtattccgtttattgaaaccagcgcaaaaacccgtcagggtgttgatgatgcattttataccctggttcgtgaaatccgcaaacataaagaaaaatga

SEQ ID NO: 4 - DNA, 1584 bp, Artificial
  Synthetic DNA
atgggcagcagccatcatcatcatcatcacagcagcggcctggtgccgcgcggcagccatatggctagcatgactggtggacagcaaatgggtcgcggatccgaaaacctgtattttcagggcgaggagcagatgaggctgcctagtgctgatgtttatagatttgcagagcctgactctgaagagaatattatatttgaagagaacatgcagcccaaggctggaattccaattatcaaagcaggaactgttattaaacttatagagaggcttacgtaccatatgtacgcagatcccaattttgttcggacatttcttacaacatacagatccttttgcaaacctcaagaactactgagtcttataatagaaaggtttgaaattccagagcctgagccaacagaagctgatcgcatagctatagagaatggagatcaacccttgagtgcagaactgaaaagatttagaaaagaatatatacagcctgtgcaactgcgagtattaaatgtatgtcggcactgggtagagcaccacttctatgattttgaaagagatgcatatcttttgcaacgaatggaagaatttattggaacagtaagaggtaaagcaatgaaaaaatgggttgaatccatcactaaaataatccaaaggaaaaaaattgcaagagacaatggaccaggtcataatattacatttcagagttcacctcccacagttgagtggcatataagcagacctgggcacatagagacttttgacctgctcaccttacacccaatagaaattgctcgacaactcactttacttgaatcagatctataccgagctgtacagccatcagaattagttggaagtgtgtggacaaaagaagacaaagaaattaactctcctaatcttctgaaaatgattcgacataccaccaacctcactctgtggtttgagaaatgtattgtagaaactgaaaatttagaagaaagagtagctgtggtgagtcgaattattgagattctacaagtctttcaagagttgaacaactttaatggtgtccttgaggttgtcagtgctatgaattcatcacctgtttacagactagaccacacatttgagcaaataccaagtcgccagaagaaaattttagaagaagctcatgaattgagtgaagatcactataagaaatatttggcaaaactcaggtctattaatccaccatgtgtgcctttctttggaatttatctcactaatatcttgaaaacagaagaaggcaaccctgaggtcctaaaaagacatggaaaagagcttataaactttagcaaaaggaggaaagtagcagaaataacaggagagatccagcagtaccaaaatcagccttactgtttacgagtagaatcagatatcaaaaggttctttgaaaacttgaatccgatgggaaatagcatggagaaggaatttacagattatcttttcaacaaatccctagaaatagaaccacgaaaccctaagcctctcccaagatttccaaaaaaatatagctatcccctaaaatctcctggtgttcgtccatcaaacccaagaccaggtacctaa